European Patent Application EP 4 660 304 A2, published December 10, 2025. Title: Fast-track Humanisation of Specific Binding Molecules. Applicant: Elasmogen Ltd. Application EP. The sequence listing filed with the application follows.

SEQUENCE LISTING (101 sequences)

SEQ ID NO: 1 - protein, 28 aa, synthetic construct
  REGION 1..28: note = Consensus sequence - humanised FW1
  SITE 1: note = misc_feature - Where X is - or D
  SITE 2: note = misc_feature - Where X is A or I or T
  SITE 3: note = misc_feature - Where X is S or Q or R
  SITE 4: note = misc_feature - Where X is V or M
  SITE 5: note = misc_feature - Where X is N or T or D
  SITE 25: note = misc_feature - Where X is L or V
  SITE 26: note = misc_feature - Where X is T or R
  SITE 27: note = misc_feature - Where X is D or G
  SITE 28: note = misc_feature - Where X is T or A or S
XXXXXQSPSSLSASVGDRVTITCVXXXX

SEQ ID NO: 2-3 - skipped (2 entries)

SEQ ID NO: 4 - protein, 20 aa, synthetic construct
  REGION 1..20: note = Consensus sequence - FW3b
  SITE 2: note = misc_feature - Where X is S or T
  SITE 4: note = misc_feature - Where X is R or T
  SITE 6: note = misc_feature - Where X is K or S or N
  SITE 7: note = misc_feature - Where X is D or S
  SITE 9: note = misc_feature - Where X is T or Q
  SITE 10: note = misc_feature - Where X is V or P
  SITE 11: note = misc_feature - Where X is A or E
  SITE 13: note = misc_feature - Where X is S or F
  SITE 14: note = misc_feature - Where X is A or G
  SITE 17: note = misc_feature - Where X is Y or R or I
  SITE 19: note = misc_feature - Where X is K or R or A
  SITE 20: note = misc_feature - Where X is A or S or L
FXLXIXXLXXXDXXTYXCXX

SEQ ID NO: 5 - skipped

SEQ ID NO: 6 - protein, 27 aa, synthetic construct
  REGION 1..27: note = Consensus sequence - V1 to V5 FW1
  SITE 1: note = misc_feature - Where X is A or T
  SITE 2: note = misc_feature - Where X is S or R
  SITE 4: note = misc_feature - Where X is N or D
  SITE 24: note = misc_feature - Where X is L or V
  SITE 26: note = misc_feature - Where X is D or G
  SITE 27: note = misc_feature - Where X is T or A
XXVXQSPSSLSASVGDRVTITCVXTXX

SEQ ID NO: 7 - protein, 28 aa, synthetic construct
  REGION 1..28: note = Consensus sequence - V6 FW1
  SITE 25: note = misc_feature - Where X is L or V
  SITE 27: note = misc_feature - Where X is D or G
  SITE 28: note = misc_feature - Where X is T or A
DIQMTQSPSSLSASVGDRVTITCVXTXX

SEQ ID NO: 8 - protein, 27 aa, synthetic construct
  REGION 1..27: note = soloMER D1v2 / C4v1 QuadX - FW1
ARVDQSPSSLSASVGDRVTITCVLRDS

SEQ ID NO: 9 - protein, 10 aa, synthetic construct
  REGION 1..10: note = Consensus sequence - V1 to V3 FW2
  SITE 2: note = misc_feature - Where X is S or Y
  SITE 4: note = misc_feature - Where X is F or Y
  SITE 10: note = misc_feature - Where X is T or S
TXWXRKNPGX

SEQ ID NO: 10 - protein, 10 aa, synthetic construct
  REGION 1..10: note = Consensus sequence - V4 to V6 FW2
  SITE 2: note = misc_feature - Where X is S or Y
  SITE 4: note = misc_feature - Where X is Y or F
  SITE 10: note = misc_feature - Where X is T or S
TXWXQQKPGX

SEQ ID NO: 11 - protein, 10 aa, synthetic construct
  REGION 1..10: note = soloMER D1v2 / C4v1 QuadX - FW2
TYWYRKKSGS

SEQ ID NO: 12 - protein, 8 aa, synthetic construct
  REGION 1..8: note = FW3a V1, V2, V3
GRYVESVN

SEQ ID NO: 13 - protein, 8 aa, synthetic construct
  REGION 1..8: note = FW3a V4, V5, V6
GRFSGSGS

SEQ ID NO: 14 - protein, 8 aa, synthetic construct
  REGION 1..8: note = soloMER D1v2 FW3a
GRYVETVN

SEQ ID NO: 15 - protein, 8 aa, synthetic construct
  REGION 1..8: note = soloMER C4v1 FW3a
GRYVETIN

SEQ ID NO: 16 - protein, 20 aa, synthetic construct
  REGION 1..20: note = Consensus sequence - FW3b
  SITE 17: note = misc_feature - Where X is Y or I
  SITE 19: note = misc_feature - Where X is K or R
FSLRIKDLTVADSATYXCXA

SEQ ID NO: 17 - protein, 20 aa, synthetic construct
  REGION 1..20: note = Consensus sequence - FW3b
  SITE 17: note = misc_feature - Where X is Y or I
  SITE 19: note = misc_feature - Where X is K or R
FTLTISSLQPEDFATYXCXA

SEQ ID NO: 18 - protein, 20 aa, synthetic construct
  REGION 1..20: note = soloMER D1v2 FW3b
FTLTISSLQPEDFATYYCAS

SEQ ID NO: 19 - protein, 20 aa, synthetic construct
  REGION 1..20: note = soloMER C4v1 Fw3b
FSLRINDLTVEDSGTYRCKL

SEQ ID NO: 20 - protein, 10 aa, synthetic construct
  REGION 1..10: note = Consensus sequence - FW4
  SITE 1: note = misc_feature - Where X is D or Y or F
  SITE 3: note = misc_feature - Where X is A or G or Q
  SITE 7: note = misc_feature - Where X is V or L
XGXGTKXEIK

SEQ ID NO: 21 - protein, 10 aa, synthetic construct
  REGION 1..10: note = soloMER D1v2 / C4v1 QuadX - FW4
YGGGTVVTVN

SEQ ID NO: 22-23 - skipped (2 entries)

SEQ ID NO: 24 - protein, 20 aa, synthetic construct
  REGION 1..20: note = Consensus sequence - FW3b
  SITE 2: note = msic_feature - Where X is S or T
  SITE 4: note = msic_feature - Where X is R or T
  SITE 6: note = msic_feature - Where X is K or S or N
  SITE 7: note = msic_feature - Where X is D or S
  SITE 9: note = msic_feature - Where X is T or Q
  SITE 10: note = msic_feature - Where X is V or P
  SITE 11: note = msic_feature - Where X is A or E
  SITE 13: note = msic_feature - Where X is S or F
  SITE 14: note = msic_feature - Where X is A or G
  SITE 17: note = msic_feature - Where X is Y or R or I
  SITE 19: note = msic_feature - Where X is K or R or A
  SITE 20: note = msic_feature - Where X is A or S or L
FXLXIXXLXXXDXXTYXCXX

SEQ ID NO: 25 - protein, 10 aa, synthetic construct
  REGION 1..10: note = Consensus sequence - FW4
  SITE 1: note = misc_feature - Where X is D or Y
XGAGTKVEIK

SEQ ID NO: 26 - skipped

SEQ ID NO: 27 - protein, 9 aa, synthetic construct
  REGION 1..9: note = Consensus sequence - HV2
  SITE 1: note = misc_feature - Where X is S or T or P
  SITE 2: note = misc_feature - Where X is N or D
  SITE 3: note = misc_feature - Where X is Q or W
  SITE 6: note = misc_feature - Where X is I or M
  SITE 9: note = misc_feature - Where X is G or S
XXXERXSIX

SEQ ID NO: 28 - skipped

SEQ ID NO: 29 - protein, 6 aa, synthetic construct
  REGION 1..6: note = CDR1 of the first VNAR domain
HCATSS

SEQ ID NO: 30 - protein, 6 aa, synthetic construct
  REGION 1..6: note = CDR1 of the second VNAR domain
NCGLSS

SEQ ID NO: 31 - protein, 6 aa, synthetic construct
  REGION 1..6: note = CDR1 of the VNAR domain
NCALSS

SEQ ID NO: 32 - protein, 9 aa, synthetic construct
  REGION 1..9: note = HV2 of the first and second VNAR domain
TNEESISKG

SEQ ID NO: 33 - protein, 5 aa, synthetic construct
  REGION 1..5: note = HV4 of the first VNAR domain
SGSKS

SEQ ID NO: 34 - protein, 5 aa, synthetic construct
  REGION 1..5: note = HV4 of the second VNAR domain
EGSKS

SEQ ID NO: 35 - protein, 11 aa, synthetic construct
  REGION 1..11: note = CDR3 of the first VNAR domain
ECQYGLAEYDV

SEQ ID NO: 36 - protein, 14 aa, synthetic construct
  REGION 1..14: note = CDR3 of the second VNAR domain
SWWTQNWRCSNSDV

SEQ ID NO: 37 - protein, 23 aa, synthetic construct
  REGION 1..23: note = CDR3 of a further VNAR domain
YIPCIDELVYMISGGTSGPIHDV

SEQ ID NO: 38 - protein, 106 aa, synthetic construct
  REGION 1..106: note = soloMER D1 QuadX v2
ARVDQSPSSLSASVGDRVTITCVLRDSHCATSSTYWYRKKSGSTNEESISKGGRYVETVNSGSKSFTLTISSLQPEDFATYYCASECQYGLAEYDVYGGGTVVTVN

SEQ ID NO: 39 - protein, 109 aa, synthetic construct
  REGION 1..109: note = soloMER DC4 QuadX v2
ARVDQSPSSLSASVGDRVTITCVLRDSNCGLSSTYWYRKKSGSTNEESISKGGRYVETINEGSKSFSLRINDLTVEDSGTYRCKLSWWTQNWRCSNSDVYGGGTVVTVN

SEQ ID NO: 40 - protein, 107 aa, synthetic construct
  REGION 1..107: note = DPK-9
DIQMTQSPSSLSASVGDRVTITCRASQSISSYLNWYQQKPGKAPKLLIYAASSLQSGVPSRFSGSGSGTDFTLTISSLQPEDFATYYCQQSYSTPNTFGQGTKVEIK

SEQ ID NO: 41 - DNA, 19 bp, synthetic construct
  misc_feature 1..19: note = Primer D3_FOR_NCoI
  source 1..19: mol_type = other DNA
agccggccatggccgcttc

SEQ ID NO: 42 - DNA, 24 bp, synthetic construct
  misc_feature 1..24: note = Primer D3_REV_NotI
  source 1..24: mol_type = other DNA
atgtgcggccgcccctgaggcctg

SEQ ID NO: 43 - protein, 106 aa, synthetic construct
  REGION 1..106: note = D1
ARVDQTPQTITKETGESLTINCVLRDSHCATSSTYWYRKKSGSTNEESISKGGRYVETVNSGSKSFSLRINDLTVEDSGTYRCASECQYGLAEYDVYGGGTVVTVN

SEQ ID NO: 44 - protein, 106 aa, synthetic construct
  REGION 1..106: note = D1-V1
ARVDQSPSSLSASVGDRVTITCVLRDSHCATSSTYWYRKKSGSTNEESISKGGRYVETVNSGSKSFSLRINDLTVEDSGTYRCASECQYGLAEYDVYGGGTKVEIK

SEQ ID NO: 45 - protein, 106 aa, synthetic construct
  REGION 1..106: note = D1-V2
ARVDQSPSSLSASVGDRVTITCVLRDSHCATSSTYWYRKKSGSTNEESISKGGRYVETVNSGSKSFTLTISSLQPEDFATYYCASECQYGLAEYDVYGGGTKVEIK

SEQ ID NO: 46 - protein, 106 aa, synthetic construct
  REGION 1..106: note = D1-V3
ARVDQSPSSLSASVGDRVTITCVLRDSHCATSSTYWYRKKPGSTNEESISKGGRFSGSGSSGSKSFTLTISSLQPEDFATYYCASECQYGLAEYDVFGQGTKVEIK

SEQ ID NO: 47 - protein, 106 aa, synthetic construct; identical to SEQ ID NO: 46
  REGION 1..106: note = D1-V4

SEQ ID NO: 48 - protein, 106 aa, synthetic construct
  REGION 1..106: note = D1-V5
ARVDQSPSSLSASVGDRVTITCVLRDSHCATSSTYWYQQKPGSTNEESISKGGRFSGSGSSGSKSFTLTISSLQPEDFATYYCASECQYGLAEYDVFGQGTKVEIK

SEQ ID NO: 49 - protein, 107 aa, synthetic construct
  REGION 1..107: note = D1-V6
DIQMTQSPSSLSASVGDRVTITCVLRDSHCATSSTYWYQQKPGSTNEESISKGGRFSGSGSSGSKSFTLTISSLQPEDFATYYCASECQYGLAEYDVFGQGTKVEIK

SEQ ID NO: 50 - protein, 109 aa, synthetic construct
  REGION 1..109: note = C4
ARVDQTPQTITKETGESLTINCVLRDSNCGLSSTYWYRKKSGSTNEESISKGGRYVETINEGSKSFSLRINDLTVEDSGTYRCKLSWWTQNWRCSNSDVYGGGTVVTVN

SEQ ID NO: 51 - protein, 109 aa, synthetic construct
  REGION 1..109: note = C4-V1
ARVDQSPSSLSASVGDRVTITCVLRDSNCGLSSTYWYRKKSGSTNEESISKGGRYVETINEGSKSFSLRINDLTVEDSGTYRCKLSWWTQNWRCSNSDVYGGGTKVEIK

SEQ ID NO: 52 - protein, 109 aa, synthetic construct
  REGION 1..109: note = C4-V2
ARVDQSPSSLSASVGDRVTITCVLRDSNCGLSSTYWYRKKSGSTNEESISKGGRYVETINEGSKSFTLTISSLQPEDFATYYCKLSWWTQNWRCSNSDVFGQGTKVEIK

SEQ ID NO: 53 - protein, 109 aa, synthetic construct
  REGION 1..109: note = C4-V3
ARVDQSPSSLSASVGDRVTITCVLRDSNCGLSSTYWYQQKPGKTNEESISKGGRYVETINEGSKSFTLTISSLQPEDFATYYCKLSWWTQNWRCSNSDVFGQGTKVEIK

SEQ ID NO: 54 - protein, 109 aa, synthetic construct
  REGION 1..109: note = C4-V4
ARVDQSPSSLSASVGDRVTITCVLRDSNCGLSSTYWYRKKSGSTNEESISKGGRFSGSGSEGSKSFTLTISSLQPEDFATYYCKLSWWTQNWRCSNSDVFGQGTKVEIK

SEQ ID NO: 55 - protein, 109 aa, synthetic construct
  REGION 1..109: note = C4-V5
ARVDQSPSSLSASVGDRVTITCVLRDSNCGLSSTYWYQQKPGSTNEESISKGGRFSGSGSEGSKSFTLTISSLQPEDFATYYCKLSWWTQNWRCSNSDVFGQGTKVEIK

SEQ ID NO: 56 - protein, 110 aa, synthetic construct
  REGION 1..110: note = C4-V6
DIQMTQSPSSLSASVGDRVTITCVLRDSNCGLSSTYWYQQKPGSTNEESISKGGRFSGSGSEGSKSFTLTISSLQPEDFATYYCKLSWWTQNWRCSNSDVFGQGTKVEIK

SEQ ID NO: 57 - protein, 140 aa, synthetic construct
  REGION 1..140: note = Consensus
ARVDQTPQTITKETGESLTINCVLRDSHCATSSTYWYRKKSGSTNEESISKGGRYVETVNSGSKSFTLTISSLQPEDFATYYCASECQYGLAEYDVYGGGTVVTVNGSGGGSGGGGSGEPKSSDKTHTCPPCPAPELLGG

SEQ ID NO: 58 - protein, 484 aa, synthetic construct
  REGION 1..484: note = soloMER D1-Fc-C4 Quad-X (NAR FW1)
ARVDQTPQTITKETGESLTINCVLRDSHCATSSTYWYRKKSGSTNEESISKGGRYVETVNSGSKSFTLTISSLQPEDFATYYCASECQYGLAEYDVYGGGTKVEIKGSGGGSGGGGSGEPKSSDKTHTCPPCPAPELLGGPSVFLFPPKPKDTLMISRTPEVTCVVVDVSHEDPEVKFNWYVDGVEVHNAKTKPREEQYNSTYRVVSVLTVLHQDWLNGKEYKCKVSNKALPAPIEKTISKAKGQPREPQVYTLPPSRDELTKNQVSLTCLVKGFYPSDIAVEWESNGQPENNYKTTPPVLDSDGSFFLYSKLTVDKSRWQQGNVFSCSVMHEALHNHYTQKSLSLSPGKGGGGSGGGGSGGGGSGGGGSGGGGSARVDQTPQTITKETGESLTINCVLRDSNCGLSSTYWYRKKSGSTNEESISKGGRYVETINEGSKSFSLRINDLTVEDSGTYRCKLSWWTQNWRCSNSDVYGGGTKVEIK

SEQ ID NO: 59 - protein, 484 aa, synthetic construct
  REGION 1..484: note = soloMER D1-Fc-C4 Quad-X (NAR FW4)-Lead
ARVDQSPSSLSASVGDRVTITCVLRDSHCATSSTYWYRKKSGSTNEESISKGGRYVETVNSGSKSFTLTISSLQPEDFATYYCASECQYGLAEYDVYGGGTVVTVNGSGGGSGGGGSGEPKSSDKTHTCPPCPAPELLGGPSVFLFPPKPKDTLMISRTPEVTCVVVDVSHEDPEVKFNWYVDGVEVHNAKTKPREEQYNSTYRVVSVLTVLHQDWLNGKEYKCKVSNKALPAPIEKTISKAKGQPREPQVYTLPPSRDELTKNQVSLTCLVKGFYPSDIAVEWESNGQPENNYKTTPPVLDSDGSFFLYSKLTVDKSRWQQGNVFSCSVMHEALHNHYTQKSLSLSPGKGGGGSGGGGSGGGGSGGGGSGGGGSARVDQSPSSLSASVGDRVTITCVLRDSNCGLSSTYWYRKKSGSTNEESISKGGRYVETINEGSKSFSLRINDLTVEDSGTYRCKLSWWTQNWRCSNSDVYGGGTVVTVN

SEQ ID NO: 60 - protein, 483 aa, synthetic construct
  REGION 1..483: note = WT D1-Fc-C4 Quad-X
ARVDQTPQTITKETGESLTINCVLRDSHCATSSTYWYRKKSGSTNEESISKGGRYVETVNSGSKSFSLRINDLTVEDSGTYRCASECQYGLAEYDVYGGGTVVTVNGSGGGSGGGGSGEPKSSDKTHTCPPCPAPELLGGPSVFLFPPKPKDTLMISRTPEVTCVVVDVSHEDPEVKFNWYVDGVEVHNAKTKPREEQYNSTYRVVSVLTVLHQDWLNGKEYKCKVSNKALPAPIEKTISKAKGQPREPQVYTLPPSRDELTKNQVSLTCLVKGFYPSDIAVEWESNGQPENNYKTTPPVLDSDGSFFLYSKLTVDKSRWQQGNVFSCSVMHEALHNHYTQKSLSLSPGKGGGGSGGGGSGGGGSGGGGSGAHSARVDQTPQTITKETGESLTINCVLRDSNCGLSSTYWYRKKSGSTNEESISKGGRYVETINEGSKSFSLRINDLTVEDSGTYRCKLSWWTQNWRCSNSDVYGGGTVVTVN

SEQ ID NO: 61 - protein, 107 aa, synthetic construct
  REGION 1..107: note = P3A1
TRVDQTPRTATKETGESLTINCVLTDTSYGLYSTSWFRKNPGTTDWERMSIGGRYVESVNKGAKSFSLRIKDLTVADSATYYCKAREARHPWLRQWYDGAGTVLTVN

SEQ ID NO: 62 - protein, 107 aa, synthetic construct
  REGION 1..107: note = P3A1 V1
TRVDQSPSSLSASVGDRVTITCVLTDTSYGLYSTSWFRKNPGTTDWERMSIGGRYVESVNKGAKSFTLTISSLQPEDFATYYCKAREARHPWLRQWYDGAGTKVEIK

SEQ ID NO: 63 - protein, 107 aa, synthetic construct
  REGION 1..107: note = P3A1 V4
TRVDQSPSSLSASVGDRVTITCVLTDTSYGLYSTSWFQQKPGTTDWERMSIGGRYSGSGSKGAKSFTLTISSLQPEDFATYYCKAREARHPWLRQWYDGAGTKVEIK

SEQ ID NO: 64 - protein, 105 aa, synthetic construct
  REGION 1..105: note = E4WT
ASVNQTPRTATKETGESLTINCVLTDTKYLYSTSWFRKNPGTTDWERMSIGGRYVESVNKGAKSFSLRIKDLTVADSATYICRAWTSFEEQVKDVYGAGTVLTVN

SEQ ID NO: 65 - protein, 105 aa, synthetic construct
  REGION 1..105: note = E4V1
ASVNQSPSSLSASVGDRVTITCVLTDTKYLYSTSWFRKNPGTTDWERMSIGGRYVESVNKGAKSFSLRIKDLTVADSATYICRAWTSFEEQVKDVYGGGTKVEIK

SEQ ID NO: 66 - protein, 105 aa, synthetic construct
  REGION 1..105: note = E4V2
ASVNQSPSSLSASVGDRVTITCVLTDTKYLYSTSWFRKNPGTTDWERMSIGGRYVESVNKGAKSFTLTISSLQPEDFATYYCRAWTSFEEQVKDVYGGGTKVEIK

SEQ ID NO: 67 - protein, 105 aa, synthetic construct
  REGION 1..105: note = E4V3
ASVNQSPSSLSASVGDRVTITCVLTDTKYLYSTSWFRKNPGTTDWERMSIGGRFSGSGSKGAKSFTLTISSLQPEDFATYYCRAWTSFEEQVKDVYGGGTKVEIK

SEQ ID NO: 68 - protein, 105 aa, synthetic construct
  REGION 1..105: note = E4V4
ASVNQSPSSLSASVGDRVTITCVLTDTKYLYSTSWYQQKPGTTDWERMSIGGRYVESVNKGAKSFTLTISSLQPEDFATYYCRAWTSFEEQVKDVYGGGTKVEIK

SEQ ID NO: 69 - protein, 105 aa, synthetic construct
  REGION 1..105: note = E4V5
ASVNQSPSSLSASVGDRVTITCVLTDTKYLYSTSWYQQKPGTTDWERMSIGGRFSGSGSKGAKSFTLTISSLQPEDFATYYCRAWTSFEEQVKDVYGGGTKVEIK

SEQ ID NO: 70 - protein, 108 aa, synthetic construct
  REGION 1..108: note = 78WT
TRVDQTPRTATKETGESLTINCVLTDTNYSLYATSWFRKNPGTTDWERMSIGGRYVESVNKGAKSFSLRIKDLTVADSATYICRAVWFPYFISDMWDVYGAGTVLTVN

SEQ ID NO: 71 - protein, 108 aa, synthetic construct
  REGION 1..108: note = 78V1
TRVDQSPSSLSASVGDRVTITCVLTDTNYSLYATSWFRKNPGTTDWERMSIGGRYVESVNKGAKSFSLRIKDLTVADSATYICRAVWFPYFISHMWDVYGGGTKVEIK

SEQ ID NO: 72 - protein, 108 aa, synthetic construct
  REGION 1..108: note = 78V2
TRVDQSPSSLSASVGDRVTITCVLTDTNYSLYATSWFRKNPGTTDWERMSIGGRYVESVNKGAKSFTLTISSLQPEDFATYYCRAVWFPYFISDMWDVYGGGTKVEIK

SEQ ID NO: 73 - protein, 108 aa, synthetic construct
  REGION 1..108: note = 78V3
TRVDQSPSSLSASVGDRVTITCVLTDTNYSLYATSWYQQKPGKTDWERMSIGGRYVESVNKGAKSFTLTISSLQPEDFATYYCRAVWFPYFISDMWDVYGGGTKVEIK

SEQ ID NO: 74 - protein, 108 aa, synthetic construct
  REGION 1..108: note = 78V4
TRVDQSPSSLSASVGDRVTITCVLTDTNYSLYATSWFRKNPGTTDWERMSIGGRFSGSGSKGAKSFTLTISSLQPEDFATYYCRAVWFPYFISDMWDVYGGGTKVEIK

SEQ ID NO: 75 - protein, 108 aa, synthetic construct
  REGION 1..108: note = 78V5
TRVDQSPSSLSASVGDRVTITCVLTDTNYSLYATSWYQQKPGKTDWERMSIGGRFSGSGSKGAKSFTLTISSLQPEDFATYYCRAVWFPYFISDMWDVYGGGTKVEIK

SEQ ID NO: 76 - protein, 105 aa, synthetic construct
  REGION 1..105: note = E4V2B09
ASVNQSPSSLSASVGDRVTITCVLTGTGYWYSTSWFRKNPGTSNEDRIIIGGRYVESVNKGTKSFTLTISSLQPEDFATYYCRAWTSFEEQVKDVYGGGTKVEIK

SEQ ID NO: 77 - protein, 105 aa, synthetic construct
  REGION 1..105: note = E4V2D10
ASVNQSPSSLSASVGDRVTITCVLTGAGYWFATSWFRKNPGTSDKESISNSGRYVESVNKRSMSFTLTISSLQPEDFATYYCRAWTSFEEQVKDVYGGGTKVEIK

SEQ ID NO: 78 - protein, 105 aa, synthetic construct
  REGION 1..105: note = E4V2F3
ASVNQSPSSLSASVGDRVTITCVLTDTNYWYSTSWFRKNPGTTNEDRIIISGRYVESVNNGPKSFTLTISSLQPEDFATYYCRAWTSFEEQVKDVYGGGTKVEIK

SEQ ID NO: 79 - protein, 105 aa, synthetic construct
  REGION 1..105: note = E4V2Cc8
ASVNQSPSSLSASVGDRVTITCVLTSAGYLYATSWFRKNPGTSDKESMIIGRRYVESVNNRSMSFTLTISSLQPEDFATYYCRAWTSFEEQVKDVYGGGTKVEIK

SEQ ID NO: 80 - protein, 105 aa, synthetic construct
  REGION 1..105: note = E4V2Cc9
ASVNQSPSSLSASVGDRVTITCVLTGTEYLYSTSWFRKNPGTPNEDRMINGGRYVESVNKGTMSFTLTISSLQPEDFATYYCRAWTSFEEQVKDVYGGGTKVEIK

SEQ ID NO: 81 - protein, 105 aa, synthetic construct
  REGION 1..105: note = E4V2Ee6
ASVNQSPSSLSASVGDRVTITCVLTDTRYLYATSWFRKNPGTTNKESISNGGRYVESVNKRSMSFTLTISSLQPEDFATYYCRAWTSFEEQVKDVYGGGTKVEIK

SEQ ID NO: 82 - protein, 105 aa, synthetic construct
  REGION 1..105: note = E4V2Ee8
ASVNQSPSSLSASVGDRVTITCVLTGASYWYSTSWFRKNPGTTDEESMSNGGRYVESVNKRPMSFTLTISSLQPEDFATYYCRAWTSFEEQVKDVYGGGTKVEIK

SEQ ID NO: 83 - protein, 105 aa, synthetic construct
  REGION 1..105: note = E4V2Gg11
ASVNQSPSSLSASVGDRVTITCVLTGTRYWFSTSWFRKNPGTTDEDSISNGGRYVESVNNGSMSFTLTISSLQPEDFATYYCRAWTSFEEQVKDVYGGGTKVEIK

SEQ ID NO: 84 - protein, 112 aa, synthetic construct
  REGION 1..112: note = D3WT
ASVNQTPRTATKETGESLTINCVLTDTSYGLYSTSWFRKNPGTTDWERMSIGGRYVESVNKRAKSFSLRIKDLTVADSATYYCKAQSGMAISTGSGHGYNWYDGAGTVLTVN

SEQ ID NO: 85 - protein, 112 aa, synthetic construct
  REGION 1..112: note = D3WT V1
ASVNQSPSSLSASVGDRVTITCVLTDTSYGLYSTSWFRKNPGTTDWERMSIGGRYVESVNKRAKSFSLRIKDLTVADSATYYCKAQSGMAISTGSGHGYNWYDGAGTKVEIK

SEQ ID NO: 86 - protein, 112 aa, synthetic construct
  REGION 1..112: note = D3WT V2
ASVNQSPSSLSASVGDRVTITCVLTDTSYGLYSTSWFRKNPGTTDWERMSIGGRYVESVNKRAKSFTLTISSLQPEDFATYYCKAQSGMAISTGSGHGYNWYDGAGTKVEIK

SEQ ID NO: 87 - protein, 112 aa, synthetic construct
  REGION 1..112: note = D3WT V4
ASVNQSPSSLSASVGDRVTITCVLTDTSYGLYSTSWYQQKPGTTDWERMSIGGRYVESVNKRAKSFTLTISSLQPEDFATYYCKAQSGMAISTGSGHGYNWYDGAGTKVEIK

SEQ ID NO: 88 - protein, 112 aa, synthetic construct
  REGION 1..112: note = D3WT V5
ASVNQSPSSLSASVGDRVTITCVLTDTSYGLYSTSWYQQKPGTTDWERMSIGGRFSGSGSKRAKSFTLTISSLQPEDFATYYCKAQSGMAISTGSGHGYNWYDGAGTKVEIK

SEQ ID NO: 89 - protein, 25 aa, synthetic construct
  REGION 1..25: note = D3V2 FW1
ASVNQSPSSLSASVGDRVTITCVLT

SEQ ID NO: 90 - protein, 8 aa, synthetic construct
  REGION 1..8: note = D3V2 CDR1
DTSYGLYS

SEQ ID NO: 91 - protein, 10 aa, synthetic construct
  REGION 1..10: note = D3V2 FW2
TSWFRKNPGT

SEQ ID NO: 92 - protein, 9 aa, synthetic construct
  REGION 1..9: note = D3V2 HV2
TDWERMSIG

SEQ ID NO: 93 - protein, 8 aa, synthetic construct
  REGION 1..8: note = D3V2 FW3a
GRYVESVN

SEQ ID NO: 94 - protein, 5 aa, synthetic construct
  REGION 1..5: note = D3V2 HV4
KRAKS

SEQ ID NO: 95 - protein, 20 aa, synthetic construct
  REGION 1..20: note = D3V2 FW3b
FTLTISSLQPEDFATYYCKA

SEQ ID NO: 96 - protein, 17 aa, synthetic construct
  REGION 1..17: note = D3V2 CDR3
QSGMAISTGSGHGYNWY

SEQ ID NO: 97 - protein, 10 aa, synthetic construct
  REGION 1..10: note = D3V2 FW4
DGAGTKVEIK

SEQ ID NO: 98 - protein, 228 aa, synthetic construct
  REGION 1..228: note = D3 V2 PAN3 F11
ASVNQSPSSLSASVGDRVTITCVLTDTNYGLYATSWFRKNPGTSNEDRIIISGRYVESVNKRTKSFTLTISSLQPEDFATYYCKAQSGMAISTGSGHGYNWYDGAGTKVEIKQASGAAAAPSVFIFPPSDEQLKSGTASVVCLLNNFYPREAKVQWKVDNALQSGNSQESVTEQDSKDSTYSLSSTLTLSKADYEKHKVYACEVTHQGLSSPVTKSFNRGESHHHHHH

SEQ ID NO: 99 - protein, 228 aa, synthetic construct
  REGION 1..228: note = D3 V2 PAN3 E08
ASVNQSPSSLSASVGDRVTITCVLTDTRYGLYSTSWFRKNPGTTDKERISIGGRYVESVNKRTKSFTLTISSLQPEDFATYYCKAQSGMAISTGSGHGYNWYDGAGTKVEIKQASGAAAAPSVFIFPPSDEQLKSGTASVVCLLNNFYPREAKVQWKVDNALQSGNSQESVTEQDSKDSTYSLSSTLTLSKADYEKHKVYACEVTHQGLSSPVTKSFNRGESHHHHHH

SEQ ID NO: 100 - protein, 228 aa, synthetic construct
  REGION 1..228: note = D3 V2 PAN F01
ASVNQSPSSLSASVGDRVTITCVLTDTKYGLYSTSWFRKNPGTTDKERISIGGRYVESVNKRTKSFTLTISSLQPEDFATYYCKAQSGMAISTGSGHGYNWYDGAGTKVEIKQASGAAAAPSVFIFPPSDEQLKSGTASVVCLLNNFYPREAKVQWKVDNALQSGNSQESVTEQDSKDSTYSLSSTLTLSKADYEKHKVYACEVTHQGLSSPVTKSFNRGESHHHHHH

SEQ ID NO: 101 - protein, 228 aa, synthetic construct
  REGION 1..228: note = D3 V2 PAN G02
ASVNQSPSSLSASVGDRVTITCVLTDTNYGLYATSWFRKNPGTTDEERMSIGGRYVESVNKRSKSFTLTISSLQPEDFATYYCKAQSGMAISTGSGHGYNWYDGAGTKVEIKQASGAAAAPSVFIFPPSDEQLKSGTASVVCLLNNFYPREAKVQWKVDNALQSGNSQESVTEQDSKDSTYSLSSTLTLSKADYEKHKVYACEVTHQGLSSPVTKSFNRGESHHHHHH